European Patent Specification EP 3 715 444 B1, published November 29, 2023. Title: LAUNDRY DETERGENT COMPOSITIONS WITH STAIN REMOVAL. Applicant: The Procter & Gamble Company The Procter & Gamble Company. The sequence listing filed with the application follows.

SEQUENCE LISTING (5 sequences)

SEQ ID NO: 1 - protein, 1050 aa, Paenibacillus sp-62047
IAGVVQSVNVSQAGYSSNDFKTATVTASDKLSDTSYQILQGTTVIATGTMKDEGYVWGKYVYSIDFSSVTATGTNFTIRSNGVSSYTFPIQTNMWNEYKDEMTAFYRLLRTTDTFAAYPAGYSNIAPSNKILHPDSFLDDAFSPDRTTHYDLTGGWFDAGDYGKYGGNQWVQGNIAISYLRHASSAAVNFDKDTNGIPDLVDEAIFGSQYLVKFANQLGGAIHNILRKGGFVLPHKVTDNVPGNTDDRALEAVEAVGGSGKSSGSLAATARAIRTAIAGGKVAANKVAQLQTLANEFQAAAIIFYNYTLTHQSGNHGSYGTMNNGGIANPLLWAEVQLYLLTGDAAYKTQAQTRINAINEAYVSSTNYWDMHPIALAEFYPVADSAIKTKIQSILKHQAYYFITLMDETPYGVLNQFGNFGVNEPHASYMADLLRYYELFNDPVALRAAKKALYWIVGNNPWNISWVSGVGSNFTDFLHTRLDEEAYSQTNTGVVLPGAMVSGPNIKDPNNKLSSSPWYEDKPIWADDTNQWRYNEYSVSIQTGLFYTIMGLSALGGNASTGGAEPVKLPITWPIIGDYVTGDVTVFAQPEGSLSNVSANGIVLSPSDGVYTTTVSTSADAPYTERKVQIKGTDDSGFTTYSNTHFTVAPALPDPSHPLLFDDFNQKGIWGSQKLDWVNWYNQNGGTASYTRTTVDTRTVGKFAHTPAATTSKAKFQPWKYNANLNGYRYLNFTMKNPGYPNTKIRIAANDGTKSVNLTSGEVAISSTWTTYQYDLNLHPTLNKSNVLIEVWLSNPTAGAYGEILIDEISAVNTNSGTAPTLSATGVNASIGNQSTVFTYTATYTDANNQAPFDVQVVIDGVIRSMTAADPTDTTYSDGRVYTYATTLPVGTHKFYFRTTDTTTNFVSTSVQTGPTVIRNKLEAEVLSINLTNYTHAVKDNADASGGKYRLFNGRQANDYIEYAVNVPKAGTYQVSARAMRLSDNGIYQLQINGSNQGTPFDTYQSSGKYLDYALGNVTITSPGTQLFRFKVTGKNASSLGYKLPLDFIQ

SEQ ID NO: 2 - protein, 1037 aa, Paenibacillus sp.
DEFDTLREKYKAMLNGGTTYNLSDPDIAARVNAITVTAQGYWDSMLKDPNRNRLWNDAPFGSDSTSITTTYRHLYDMALAYTTYGSSLQGNAALKADIISGLDWMNANQFYNGCSQYQNWWHWQIGGPMALNDIVALMYTELTATQISNYMAAIYYTQASVTMTGANRLWESQVIAISGILNKDSARVAAGRDGISALLPYVAKGDGFYNDGSFVQHTYYAYNGGYGSELLSGIADLIFILNGSSWQVTDPNKNNVYRWIYDSYEPFIYKGNLMDMVRGREISRHGLQDDKAAVTVMASIIRLSQTAASADATAFKRMVKYWLLLDTDKTFLKAVSIDLIIAANQLVNDSTVTSRGELVKYKQFSGMDRAVQLRPGFGFGLSMFSSRIGNYESINAENNKGWHTGDGMTYLYNTDLSQFNDHFWATVDNYRLPGTTVLQNTTQTANSRSDKSWAGGTDILGQYGVSGMELHTVGKSLTAKKSWFMFDDEIVALGSGIASTDGIATETIVENRKLNSSGNNALIVNGTAKPGSLGWSETMTGTNYIHLAGSVPGSDIGYYFPGGAAVKGLREARSGSWSSLNSSASWKDSTLHTRNFMTLWFDHGMNPTNGSYSYVLLPNKTSSAVASYAATPQISILENSSSAQAVKETQLNVTGINFWNDEPTTVGLVTSNRKASVMTKETASDFEISVSDPTQSNVGTIYIDVNKSATGLISKDNEITVIQYYPTMKFKVNVNNSGGKSYKVKFSLTGTPGSNPSPIPIPNPYEAEALPINALTDTPVVYNDANASGGKKLGFNNNAVDDYVEFSLDVTQPGTYDVKSRIMKSTNSGIYQLSINGTNVGSAQDMFWTTSELSKEFTMGSYSFSTPGSYLFRLKTTGKNVSSSGYKLMLDNFSLVSTGIDTTVIVDNADAAGVTKVGTWTGTNTQTDRYGADYIHDGNTGKGTKSVTFTPNVPISGTYQVYMMWAAHTNRATNVPVDVTHSGGTATLNVNQQGNGGVWNLLGTYSFNAGSTGAIKIRTDATNGYVVADAVKLVKVP

SEQ ID NO: 3 - protein, 490 aa, Bacillus hemicellulosilyticus
MRNFGKLIVSSCLLFSFFLFASDGHSQTHSGFYIEGSTLYDANGEPFVMRGINHGHAWYKHDSNVAIPAIANQGANTIRIVLSDGGQWAKDDINTLNQVLDLAEEHEMIAVVEVHDATGSNSMADLNRAVDYWIEMKDALIGKEDRVIINIANEWYGAWDGQGWANGYKEVIPRLRNAGFTHTLMVDAAGWGQYPQSIHDYGQEVFNADPLANTMFSIHMYEYAGGNASMVQSNIDGVVDQGLALVIGEFGHMHTDGDVDEATILSYSQQRGVGWLAWSWKGNGTQWEYLDLSYDWQGTNLTSWGNTIVHGPNGLLETSIPSSIFHTAPNNGDPPPHNGNETILYDFEHGTQGWSGSSLLGGPWTTNEWSTNGNHSLKADIFLSANSKHELAKVENRNLSGYSTLQATVRHAHWGNVGNLTARMYVKTGSNYSWFNGDPIPVNSANGTTVTLPLSSIPNLNDVKEIGVEFIGASNSNGQTAIYLDHVTIQ

SEQ ID NO: 4 - protein, 297 aa, Paenibacillus sp.
MATGFYVSGNKLYDSTGKPFVMRGVNHGHSWFKNDLNTAIPAIAKTGANTVRIVLSNGSLYTKDDLNAVKNIINVVNQNKMIAVLEVHDATGKDDYNSLDAAVNYWISIKEALIGKEDRVIVNIANEWYGTWNGSAWADGYKKAIPKLRNAGIKNTLIVDAAGWGQFPQSIVDYGQSVFAADSQKNTVFSIHMYEYAGKDAATVKANMENVLNKGLALIIGEFGGYHTNGDVDEYAIMRYGQEKGVGWLAWSWYGNSSGLNYLDMATGPNGSLTSFGNTVVNDTYGIKNTSQKAGIF

SEQ ID NO: 5 - protein, 269 aa, Thermomyces lanuginosus [sequence omitted]